European Patent Application EP 4 474 396 A1, published December 11, 2024. Title: USE OF CCL11. Applicant: NEWISH TECHNOLOGY (BEIJING) CO., LTD. The sequence listing filed with the application follows.

SEQUENCE LISTING (17 sequences)

SEQ ID NO: 1 - protein, 157 aa, Artificial sequence
  E6 protein of HPV16
HQKRTAMFQDPQERPRKLPQLCTELQTTIHDIILECVYCKQQLLRREVYDFAFRDLCIVYRDGNPYAVGDKCLKFYSKISEYRHYCYSLYGTTLEQQYNKPLCDLLIRCINCQKPLCPEEKQRHLDKKQRFHNTRGRWTGRCMSCCRSSRTRRETQL

SEQ ID NO: 2 - protein, 100 aa, Artificial sequence
  E7 protein of HPV16
HGDTPTLHEYMLDLQPETTDLYCGSGYEQLNDSSEEEDEIDGPAGQAEPDRAHYNIVTFCCKCDSTLRLCVQSTHVDIRTLEDLLMGTLGIVCPICSQKP

SEQ ID NO: 3 - protein, 74 aa, Artificial sequence
  CCL11
GPASVPTTCCFNLANRKIPLQRLESYRRITSGKCPQKAVIFKTKLAKDICADPKKKWVQDSMKYLDQKSPTPKP

SEQ ID NO: 4 - protein, 31 aa, Artificial sequence
  T2 fragment
PGSGYIPEAPRDGQAYVRKDGEWVLLSTFLG

SEQ ID NO: 5 - protein, 18 aa, Artificial sequence
  IgE signal peptide
MDWTWILFLVAAATRVHS

SEQ ID NO: 6 - DNA, 4556 bp, Artificial sequence
  pVR-CCL11-E6E7-T2
gactcttcgcgatgtacgggccagatatacgcgttccattgcatacgttgtatccatatcataatatgtacatttatattggctcatgtccaacattaccgccatgttgacattgattattgactagttattaatagtaatcaattacggggtcattagttcatagcccatatatggagttccgcgttacataacttacggtaaatggcccgcctggctgaccgcccaacgacccccgcccattgacgtcaataatgacgtatgttcccatagtaacgccaatagggactttccattgacgtcaatgggtggagtatttacggtaaactgcccacttggcagtacatcaagtgtatcatatgccaagtacgccccctattgacgtcaatgacggtaaatggcccgcctggcattatgcccagtacatgaccttatgggactttcctacttggcagtacatctacgtattagtcatcgctattaccatggtgatgcggttttggcagtacatcaatgggcgtggatagcggtttgactcacggggatttccaagtctccaccccattgacgtcaatgggagtttgttttggcaccaaaatcaacgggactttccaaaatgtcgtaacaactccgccccattgacgcaaatgggcggtaggcgtgtacggtgggaggtctatataagcagagctcgtttagtgaaccgtcagatcgcctggagacgccatccacgctgttttgacctccatagaagacaccgggaccgatccagcctccatcggctcgcatctctccttcacgcgcccgccgccctacctgaggccgccatccacgccggttgagtcgcgttctgccgcctcccgcctgtggtgcctcctgaactgcgtccgccgtctaggtaagtttaaagctcaggtcgagaccgggcctttgtccggcgctcccttggagcctacctagactcagccggctctccacgctttgcctgaccctgcttgctcaactctactctggctaactagagaacccactgcttactggcttatcgaaattaatacgactcactatagggagacccaagctggctagcgtttaaacttaagcttggtaccgagctcggatccgccaccatggactggacctggatcctgttcctggtggccgccgccacaagggtgcacagcgggccagcttctgtcccaaccacctgctgctttaacctggccaataggaagataccccttcagcgactagagagctacaggagaatcaccagtggcaaatgtccccagaaagctgtgatcttcaagaccaaactggccaaggatatctgtgccgaccccaagaagaagtgggtgcaggattccatgaagtatctggaccaaaaatctccaactccaaagccaggaggaggaggagggagcggaggaggaggcggacaccagaagaggacagcaatgttccaggacccacaggagaggccaaggaagctgccacagctgtgcacagagctgcagacaacaatccacgatattatcctggagtgcgtgtattgcaagcagcagctgctgaggagggaggtgtatgacttcgctttcagagacctgtgtatcgtgtaccgggacgggaacccttacgcagtgggcgacaagtgcctgaagttctatagcaagatcagcgagtacaggcactactgttacagcctgtatggaaccaccctggagcagcagtataacaaacctctgtgcgacctgctgatcaggtgcatcaactgccagaagcccctgtgccccgaggagaagcagagacacctggacaagaagcagaggttccacaataccaggggccgctggaccggccgctgcatgtcttgctgcaggtccagccggaccaggagagagacccagctggccggagcacacggagatacacccaccctgcacgagtacatgctggacctgcagcctgagaccaccgacctgtactgcgggagtggatacgaacagctgaacgacagcagcgaggaggaggacgagatcgacggccccgccggacaggctgagcctgatagggcccactacaacattgtgacattttgctgcaagtgcgacagcaccctgaggctgtgcgtgcagagcacccacgtggatatcaggaccctggaggatctgctgatgggaaccctgggcatcgtgtgccccatctgctcccagaagcctcctggatctggctacattcctgaagcccctcgcgacggccaggcctacgtgagaaaagacggcgaatgggtgctgctgagcacctttctgggcgactacaaggacgacgacgacaagtgatgactcgagtctagagggcccgtttaaacccgctgatcagcctcgactgtgccttctagttgccagccatctgttgtttgcccctcccccgtgccttccttgaccctggaaggtgccactcccactgtcctttcctaataaaatgaggaaattgcatcgcattgtctgagtaggtgtcattctattctggggggtggggtggggcaggacagcaagggggaggattgggaagacaatagcaggcatgctggggatgcggtgggctctatggcttctactgggcggttttatggacagcaagcgaaccggaattgccagctggggcgccctctggtaaggttgggaagccctgcaaagtaaactggatggctttctcgccgccaaggatctgatggcgcaggggatcaagctctgatcaagagacaggatgaggatcgtttcgcatgattgaacaagatggattgcacgcaggttctccggccgcttgggtggagaggctattcggctatgactgggcacaacagacaatcggctgctctgatgccgccgtgttccggctgtcagcgcaggggcgcccggttctttttgtcaagaccgacctgtccggtgccctgaatgaactgcaagacgaggcagcgcggctatcgtggctggccacgacgggcgttccttgcgcagctgtgctcgacgttgtcactgaagcgggaagggactggctgctattgggcgaagtgccggggcaggatctcctgtcatctcaccttgctcctgccgagaaagtatccatcatggctgatgcaatgcggcggctgcatacgcttgatccggctacctgcccattcgaccaccaagcgaaacatcgcatcgagcgagcacgtactcggatggaagccggtcttgtcgatcaggatgatctggacgaagagcatcaggggctcgcgccagccgaactgttcgccaggctcaaggcgagcatgcccgacggcgaggatctcgtcgtgacccatggcgatgcctgcttgccgaatatcatggtggaaaatggccgcttttctggattcatcgactgtggccggctgggtgtggcggaccgctatcaggacatagcgttggctacccgtgatattgctgaagagcttggcggcgaatgggctgaccgcttcctcgtgctttacggtatcgccgctcccgattcgcagcgcatcgccttctatcgccttcttgacgagttcttctgaattattaacgcttacaatttcctgatgcggtattttctccttacgcatctgtgcggtatttcacaccgcatacaggtggcacttttcggggaaatgtgcgcggaacccctatttgtttatttttctaaatacattcaaatatgtatccgctcatgagacaataaccctgataaatgcttcaataatagcacgtgctaaaacttcatttttaatttaaaaggatctaggtgaagatcctttttgataatctcatgaccaaaatcccttaacgtgagttttcgttccactgagcgtcagaccccgtagaaaagatcaaaggatcttcttgagatcctttttttctgcgcgtaatctgctgcttgcaaacaaaaaaaccaccgctaccagcggtggtttgtttgccggatcaagagctaccaactctttttccgaaggtaactggcttcagcagagcgcagataccaaatactgtccttctagtgtagccgtagttaggccaccacttcaagaactctgtagcaccgcctacatacctcgctctgctaatcctgttaccagtggctgctgccagtggcgataagtcgtgtcttaccgggttggactcaagacgatagttaccggataaggcgcagcggtcgggctgaacggggggttcgtgcacacagcccagcttggagcgaacgacctacaccgaactgagatacctacagcgtgagctatgagaaagcgccacgcttcccgaagggagaaaggcggacaggtatccggtaagcggcagggtcggaacaggagagcgcacgagggagcttccagggggaaacgcctggtatctttatagtcctgtcgggtttcgccacctctgacttgagcgtcgatttttgtgatgctcgtcaggggggcggagcctatggaaaaacgccagcaacgcggcctttttacggttcctgggcttttgctggccttttgctcacatgttctt

SEQ ID NO: 7 - DNA, 4463 bp, Artificial sequence
  pVR-CCL11-E6E7
gactcttcgcgatgtacgggccagatatacgcgttccattgcatacgttgtatccatatcataatatgtacatttatattggctcatgtccaacattaccgccatgttgacattgattattgactagttattaatagtaatcaattacggggtcattagttcatagcccatatatggagttccgcgttacataacttacggtaaatggcccgcctggctgaccgcccaacgacccccgcccattgacgtcaataatgacgtatgttcccatagtaacgccaatagggactttccattgacgtcaatgggtggagtatttacggtaaactgcccacttggcagtacatcaagtgtatcatatgccaagtacgccccctattgacgtcaatgacggtaaatggcccgcctggcattatgcccagtacatgaccttatgggactttcctacttggcagtacatctacgtattagtcatcgctattaccatggtgatgcggttttggcagtacatcaatgggcgtggatagcggtttgactcacggggatttccaagtctccaccccattgacgtcaatgggagtttgttttggcaccaaaatcaacgggactttccaaaatgtcgtaacaactccgccccattgacgcaaatgggcggtaggcgtgtacggtgggaggtctatataagcagagctcgtttagtgaaccgtcagatcgcctggagacgccatccacgctgttttgacctccatagaagacaccgggaccgatccagcctccatcggctcgcatctctccttcacgcgcccgccgccctacctgaggccgccatccacgccggttgagtcgcgttctgccgcctcccgcctgtggtgcctcctgaactgcgtccgccgtctaggtaagtttaaagctcaggtcgagaccgggcctttgtccggcgctcccttggagcctacctagactcagccggctctccacgctttgcctgaccctgcttgctcaactctactctggctaactagagaacccactgcttactggcttatcgaaattaatacgactcactatagggagacccaagctggctagcgtttaaacttaagcttggtaccgagctcggatccgccaccatggactggacctggatcctgttcctggtggccgccgccacaagggtgcacagcgggccagcttctgtcccaaccacctgctgctttaacctggccaataggaagataccccttcagcgactagagagctacaggagaatcaccagtggcaaatgtccccagaaagctgtgatcttcaagaccaaactggccaaggatatctgtgccgaccccaagaagaagtgggtgcaggattccatgaagtatctggaccaaaaatctccaactccaaagccaggaggaggaggagggagcggaggaggaggcggacaccagaagaggacagcaatgttccaggacccacaggagaggccaaggaagctgccacagctgtgcacagagctgcagacaacaatccacgatattatcctggagtgcgtgtattgcaagcagcagctgctgaggagggaggtgtatgacttcgctttcagagacctgtgtatcgtgtaccgggacgggaacccttacgcagtgggcgacaagtgcctgaagttctatagcaagatcagcgagtacaggcactactgttacagcctgtatggaaccaccctggagcagcagtataacaaacctctgtgcgacctgctgatcaggtgcatcaactgccagaagcccctgtgccccgaggagaagcagagacacctggacaagaagcagaggttccacaataccaggggccgctggaccggccgctgcatgtcttgctgcaggtccagccggaccaggagagagacccagctggccggagcacacggagatacacccaccctgcacgagtacatgctggacctgcagcctgagaccaccgacctgtactgcgggagtggatacgaacagctgaacgacagcagcgaggaggaggacgagatcgacggccccgccggacaggctgagcctgatagggcccactacaacattgtgacattttgctgcaagtgcgacagcaccctgaggctgtgcgtgcagagcacccacgtggatatcaggaccctggaggatctgctgatgggaaccctgggcatcgtgtgccccatctgctcccagaagcctgactacaaggacgacgacgacaagtgatgactcgagtctagagggcccgtttaaacccgctgatcagcctcgactgtgccttctagttgccagccatctgttgtttgcccctcccccgtgccttccttgaccctggaaggtgccactcccactgtcctttcctaataaaatgaggaaattgcatcgcattgtctgagtaggtgtcattctattctggggggtggggtggggcaggacagcaagggggaggattgggaagacaatagcaggcatgctggggatgcggtgggctctatggcttctactgggcggttttatggacagcaagcgaaccggaattgccagctggggcgccctctggtaaggttgggaagccctgcaaagtaaactggatggctttctcgccgccaaggatctgatggcgcaggggatcaagctctgatcaagagacaggatgaggatcgtttcgcatgattgaacaagatggattgcacgcaggttctccggccgcttgggtggagaggctattcggctatgactgggcacaacagacaatcggctgctctgatgccgccgtgttccggctgtcagcgcaggggcgcccggttctttttgtcaagaccgacctgtccggtgccctgaatgaactgcaagacgaggcagcgcggctatcgtggctggccacgacgggcgttccttgcgcagctgtgctcgacgttgtcactgaagcgggaagggactggctgctattgggcgaagtgccggggcaggatctcctgtcatctcaccttgctcctgccgagaaagtatccatcatggctgatgcaatgcggcggctgcatacgcttgatccggctacctgcccattcgaccaccaagcgaaacatcgcatcgagcgagcacgtactcggatggaagccggtcttgtcgatcaggatgatctggacgaagagcatcaggggctcgcgccagccgaactgttcgccaggctcaaggcgagcatgcccgacggcgaggatctcgtcgtgacccatggcgatgcctgcttgccgaatatcatggtggaaaatggccgcttttctggattcatcgactgtggccggctgggtgtggcggaccgctatcaggacatagcgttggctacccgtgatattgctgaagagcttggcggcgaatgggctgaccgcttcctcgtgctttacggtatcgccgctcccgattcgcagcgcatcgccttctatcgccttcttgacgagttcttctgaattattaacgcttacaatttcctgatgcggtattttctccttacgcatctgtgcggtatttcacaccgcatacaggtggcacttttcggggaaatgtgcgcggaacccctatttgtttatttttctaaatacattcaaatatgtatccgctcatgagacaataaccctgataaatgcttcaataatagcacgtgctaaaacttcatttttaatttaaaaggatctaggtgaagatcctttttgataatctcatgaccaaaatcccttaacgtgagttttcgttccactgagcgtcagaccccgtagaaaagatcaaaggatcttcttgagatcctttttttctgcgcgtaatctgctgcttgcaaacaaaaaaaccaccgctaccagcggtggtttgtttgccggatcaagagctaccaactctttttccgaaggtaactggcttcagcagagcgcagataccaaatactgtccttctagtgtagccgtagttaggccaccacttcaagaactctgtagcaccgcctacatacctcgctctgctaatcctgttaccagtggctgctgccagtggcgataagtcgtgtcttaccgggttggactcaagacgatagttaccggataaggcgcagcggtcgggctgaacggggggttcgtgcacacagcccagcttggagcgaacgacctacaccgaactgagatacctacagcgtgagctatgagaaagcgccacgcttcccgaagggagaaaggcggacaggtatccggtaagcggcagggtcggaacaggagagcgcacgagggagcttccagggggaaacgcctggtatctttatagtcctgtcgggtttcgccacctctgacttgagcgtcgatttttgtgatgctcgtcaggggggcggagcctatggaaaaacgccagcaacgcggcctttttacggttcctgggcttttgctggccttttgctcacatgttctt

SEQ ID NO: 8 - DNA, 4157 bp, Artificial sequence
  pVR-E6E7
gactcttcgcgatgtacgggccagatatacgcgttccattgcatacgttgtatccatatcataatatgtacatttatattggctcatgtccaacattaccgccatgttgacattgattattgactagttattaatagtaatcaattacggggtcattagttcatagcccatatatggagttccgcgttacataacttacggtaaatggcccgcctggctgaccgcccaacgacccccgcccattgacgtcaataatgacgtatgttcccatagtaacgccaatagggactttccattgacgtcaatgggtggagtatttacggtaaactgcccacttggcagtacatcaagtgtatcatatgccaagtacgccccctattgacgtcaatgacggtaaatggcccgcctggcattatgcccagtacatgaccttatgggactttcctacttggcagtacatctacgtattagtcatcgctattaccatggtgatgcggttttggcagtacatcaatgggcgtggatagcggtttgactcacggggatttccaagtctccaccccattgacgtcaatgggagtttgttttggcaccaaaatcaacgggactttccaaaatgtcgtaacaactccgccccattgacgcaaatgggcggtaggcgtgtacggtgggaggtctatataagcagagctcgtttagtgaaccgtcagatcgcctggagacgccatccacgctgttttgacctccatagaagacaccgggaccgatccagcctccatcggctcgcatctctccttcacgcgcccgccgccctacctgaggccgccatccacgccggttgagtcgcgttctgccgcctcccgcctgtggtgcctcctgaactgcgtccgccgtctaggtaagtttaaagctcaggtcgagaccgggcctttgtccggcgctcccttggagcctacctagactcagccggctctccacgctttgcctgaccctgcttgctcaactctactctggctaactagagaacccactgcttactggcttatcgaaattaatacgactcactatagggagacccaagctggctagcgtttaaacttaagcttggtaccgagctcggatccgccaccatgcaccagaagaggacagcaatgttccaggacccacaggagaggccaaggaagctgccacagctgtgcacagagctgcagacaacaatccacgatattatcctggagtgcgtgtattgcaagcagcagctgctgaggagggaggtgtatgacttcgctttcagagacctgtgtatcgtgtaccgggacgggaacccttacgcagtgggcgacaagtgcctgaagttctatagcaagatcagcgagtacaggcactactgttacagcctgtatggaaccaccctggagcagcagtataacaaacctctgtgcgacctgctgatcaggtgcatcaactgccagaagcccctgtgccccgaggagaagcagagacacctggacaagaagcagaggttccacaataccaggggccgctggaccggccgctgcatgtcttgctgcaggtccagccggaccaggagagagacccagctggccggagcacacggagatacacccaccctgcacgagtacatgctggacctgcagcctgagaccaccgacctgtactgcgggagtggatacgaacagctgaacgacagcagcgaggaggaggacgagatcgacggccccgccggacaggctgagcctgatagggcccactacaacattgtgacattttgctgcaagtgcgacagcaccctgaggctgtgcgtgcagagcacccacgtggatatcaggaccctggaggatctgctgatgggaaccctgggcatcgtgtgccccatctgctcccagaagcctgactacaaggacgacgacgacaagtgatgactcgagtctagagggcccgtttaaacccgctgatcagcctcgactgtgccttctagttgccagccatctgttgtttgcccctcccccgtgccttccttgaccctggaaggtgccactcccactgtcctttcctaataaaatgaggaaattgcatcgcattgtctgagtaggtgtcattctattctggggggtggggtggggcaggacagcaagggggaggattgggaagacaatagcaggcatgctggggatgcggtgggctctatggcttctactgggcggttttatggacagcaagcgaaccggaattgccagctggggcgccctctggtaaggttgggaagccctgcaaagtaaactggatggctttctcgccgccaaggatctgatggcgcaggggatcaagctctgatcaagagacaggatgaggatcgtttcgcatgattgaacaagatggattgcacgcaggttctccggccgcttgggtggagaggctattcggctatgactgggcacaacagacaatcggctgctctgatgccgccgtgttccggctgtcagcgcaggggcgcccggttctttttgtcaagaccgacctgtccggtgccctgaatgaactgcaagacgaggcagcgcggctatcgtggctggccacgacgggcgttccttgcgcagctgtgctcgacgttgtcactgaagcgggaagggactggctgctattgggcgaagtgccggggcaggatctcctgtcatctcaccttgctcctgccgagaaagtatccatcatggctgatgcaatgcggcggctgcatacgcttgatccggctacctgcccattcgaccaccaagcgaaacatcgcatcgagcgagcacgtactcggatggaagccggtcttgtcgatcaggatgatctggacgaagagcatcaggggctcgcgccagccgaactgttcgccaggctcaaggcgagcatgcccgacggcgaggatctcgtcgtgacccatggcgatgcctgcttgccgaatatcatggtggaaaatggccgcttttctggattcatcgactgtggccggctgggtgtggcggaccgctatcaggacatagcgttggctacccgtgatattgctgaagagcttggcggcgaatgggctgaccgcttcctcgtgctttacggtatcgccgctcccgattcgcagcgcatcgccttctatcgccttcttgacgagttcttctgaattattaacgcttacaatttcctgatgcggtattttctccttacgcatctgtgcggtatttcacaccgcatacaggtggcacttttcggggaaatgtgcgcggaacccctatttgtttatttttctaaatacattcaaatatgtatccgctcatgagacaataaccctgataaatgcttcaataatagcacgtgctaaaacttcatttttaatttaaaaggatctaggtgaagatcctttttgataatctcatgaccaaaatcccttaacgtgagttttcgttccactgagcgtcagaccccgtagaaaagatcaaaggatcttcttgagatcctttttttctgcgcgtaatctgctgcttgcaaacaaaaaaaccaccgctaccagcggtggtttgtttgccggatcaagagctaccaactctttttccgaaggtaactggcttcagcagagcgcagataccaaatactgtccttctagtgtagccgtagttaggccaccacttcaagaactctgtagcaccgcctacatacctcgctctgctaatcctgttaccagtggctgctgccagtggcgataagtcgtgtcttaccgggttggactcaagacgatagttaccggataaggcgcagcggtcgggctgaacggggggttcgtgcacacagcccagcttggagcgaacgacctacaccgaactgagatacctacagcgtgagctatgagaaagcgccacgcttcccgaagggagaaaggcggacaggtatccggtaagcggcagggtcggaacaggagagcgcacgagggagcttccagggggaaacgcctggtatctttatagtcctgtcgggtttcgccacctctgacttgagcgtcgatttttgtgatgctcgtcaggggggcggagcctatggaaaaacgccagcaacgcggcctttttacggttcctgggcttttgctggccttttgctcacatgttctt

SEQ ID NO: 9 - DNA, 1206 bp, Artificial sequence
  fusion protein in plasmid pVR-CCL11-E6E7-T2
atggactggacctggatcctgttcctggtggccgccgccacaagggtgcacagcgggccagcttctgtcccaaccacctgctgctttaacctggccaataggaagataccccttcagcgactagagagctacaggagaatcaccagtggcaaatgtccccagaaagctgtgatcttcaagaccaaactggccaaggatatctgtgccgaccccaagaagaagtgggtgcaggattccatgaagtatctggaccaaaaatctccaactccaaagccaggaggaggaggagggagcggaggaggaggcggacaccagaagaggacagcaatgttccaggacccacaggagaggccaaggaagctgccacagctgtgcacagagctgcagacaacaatccacgatattatcctggagtgcgtgtattgcaagcagcagctgctgaggagggaggtgtatgacttcgctttcagagacctgtgtatcgtgtaccgggacgggaacccttacgcagtgggcgacaagtgcctgaagttctatagcaagatcagcgagtacaggcactactgttacagcctgtatggaaccaccctggagcagcagtataacaaacctctgtgcgacctgctgatcaggtgcatcaactgccagaagcccctgtgccccgaggagaagcagagacacctggacaagaagcagaggttccacaataccaggggccgctggaccggccgctgcatgtcttgctgcaggtccagccggaccaggagagagacccagctggccggagcacacggagatacacccaccctgcacgagtacatgctggacctgcagcctgagaccaccgacctgtactgcgggagtggatacgaacagctgaacgacagcagcgaggaggaggacgagatcgacggccccgccggacaggctgagcctgatagggcccactacaacattgtgacattttgctgcaagtgcgacagcaccctgaggctgtgcgtgcagagcacccacgtggatatcaggaccctggaggatctgctgatgggaaccctgggcatcgtgtgccccatctgctcccagaagcctcctggatctggctacattcctgaagcccctcgcgacggccaggcctacgtgagaaaagacggcgaatgggtgctgctgagcacctttctgggcgactacaaggacgacgacgacaag

SEQ ID NO: 10 - DNA, 1113 bp, Artificial sequence
  fusion protein in plasmid pVR-CCL11-E6E7
atggactggacctggatcctgttcctggtggccgccgccacaagggtgcacagcgggccagcttctgtcccaaccacctgctgctttaacctggccaataggaagataccccttcagcgactagagagctacaggagaatcaccagtggcaaatgtccccagaaagctgtgatcttcaagaccaaactggccaaggatatctgtgccgaccccaagaagaagtgggtgcaggattccatgaagtatctggaccaaaaatctccaactccaaagccaggaggaggaggagggagcggaggaggaggcggacaccagaagaggacagcaatgttccaggacccacaggagaggccaaggaagctgccacagctgtgcacagagctgcagacaacaatccacgatattatcctggagtgcgtgtattgcaagcagcagctgctgaggagggaggtgtatgacttcgctttcagagacctgtgtatcgtgtaccgggacgggaacccttacgcagtgggcgacaagtgcctgaagttctatagcaagatcagcgagtacaggcactactgttacagcctgtatggaaccaccctggagcagcagtataacaaacctctgtgcgacctgctgatcaggtgcatcaactgccagaagcccctgtgccccgaggagaagcagagacacctggacaagaagcagaggttccacaataccaggggccgctggaccggccgctgcatgtcttgctgcaggtccagccggaccaggagagagacccagctggccggagcacacggagatacacccaccctgcacgagtacatgctggacctgcagcctgagaccaccgacctgtactgcgggagtggatacgaacagctgaacgacagcagcgaggaggaggacgagatcgacggccccgccggacaggctgagcctgatagggcccactacaacattgtgacattttgctgcaagtgcgacagcaccctgaggctgtgcgtgcagagcacccacgtggatatcaggaccctggaggatctgctgatgggaaccctgggcatcgtgtgccccatctgctcccagaagcctgactacaaggacgacgacgacaag

SEQ ID NO: 11 - DNA, 807 bp, Artificial sequence
  fusion protein in plasmid pVR-E6E7
atgcaccagaagaggacagcaatgttccaggacccacaggagaggccaaggaagctgccacagctgtgcacagagctgcagacaacaatccacgatattatcctggagtgcgtgtattgcaagcagcagctgctgaggagggaggtgtatgacttcgctttcagagacctgtgtatcgtgtaccgggacgggaacccttacgcagtgggcgacaagtgcctgaagttctatagcaagatcagcgagtacaggcactactgttacagcctgtatggaaccaccctggagcagcagtataacaaacctctgtgcgacctgctgatcaggtgcatcaactgccagaagcccctgtgccccgaggagaagcagagacacctggacaagaagcagaggttccacaataccaggggccgctggaccggccgctgcatgtcttgctgcaggtccagccggaccaggagagagacccagctggccggagcacacggagatacacccaccctgcacgagtacatgctggacctgcagcctgagaccaccgacctgtactgcgggagtggatacgaacagctgaacgacagcagcgaggaggaggacgagatcgacggccccgccggacaggctgagcctgatagggcccactacaacattgtgacattttgctgcaagtgcgacagcaccctgaggctgtgcgtgcagagcacccacgtggatatcaggaccctggaggatctgctgatgggaaccctgggcatcgtgtgccccatctgctcccagaagcctgactacaaggacgacgacgacaag

SEQ ID NO: 12 - RNA, 1206 nt, Artificial sequence
  fusion protein in plasmid pVR-CCL11-E6E7-T2
auggacuggaccuggauccuguuccugguggccgccgccacaagggugcacagcgggccagcuucugucccaaccaccugcugcuuuaaccuggccaauaggaagauaccccuucagcgacuagagagcuacaggagaaucaccaguggcaaauguccccagaaagcugugaucuucaagaccaaacuggccaaggauaucugugccgaccccaagaagaagugggugcaggauuccaugaaguaucuggaccaaaaaucuccaacuccaaagccaggaggaggaggagggagcggaggaggaggcggacaccagaagaggacagcaauguuccaggacccacaggagaggccaaggaagcugccacagcugugcacagagcugcagacaacaauccacgauauuauccuggagugcguguauugcaagcagcagcugcugaggagggagguguaugacuucgcuuucagagaccuguguaucguguaccgggacgggaacccuuacgcagugggcgacaagugccugaaguucuauagcaagaucagcgaguacaggcacuacuguuacagccuguauggaaccacccuggagcagcaguauaacaaaccucugugcgaccugcugaucaggugcaucaacugccagaagccccugugccccgaggagaagcagagacaccuggacaagaagcagagguuccacaauaccaggggccgcuggaccggccgcugcaugucuugcugcagguccagccggaccaggagagagacccagcuggccggagcacacggagauacacccacccugcacgaguacaugcuggaccugcagccugagaccaccgaccuguacugcgggaguggauacgaacagcugaacgacagcagcgaggaggaggacgagaucgacggccccgccggacaggcugagccugauagggcccacuacaacauugugacauuuugcugcaagugcgacagcacccugaggcugugcgugcagagcacccacguggauaucaggacccuggaggaucugcugaugggaacccugggcaucgugugccccaucugcucccagaagccuccuggaucuggcuacauuccugaagccccucgcgacggccaggccuacgugagaaaagacggcgaaugggugcugcugagcaccuuucugggcgacuacaaggacgacgacgacaag

SEQ ID NO: 13 - RNA, 1113 nt, Artificial sequence
  fusion protein in plasmid pVR-CCL11-E6E7
auggacuggaccuggauccuguuccugguggccgccgccacaagggugcacagcgggccagcuucugucccaaccaccugcugcuuuaaccuggccaauaggaagauaccccuucagcgacuagagagcuacaggagaaucaccaguggcaaauguccccagaaagcugugaucuucaagaccaaacuggccaaggauaucugugccgaccccaagaagaagugggugcaggauuccaugaaguaucuggaccaaaaaucuccaacuccaaagccaggaggaggaggagggagcggaggaggaggcggacaccagaagaggacagcaauguuccaggacccacaggagaggccaaggaagcugccacagcugugcacagagcugcagacaacaauccacgauauuauccuggagugcguguauugcaagcagcagcugcugaggagggagguguaugacuucgcuuucagagaccuguguaucguguaccgggacgggaacccuuacgcagugggcgacaagugccugaaguucuauagcaagaucagcgaguacaggcacuacuguuacagccuguauggaaccacccuggagcagcaguauaacaaaccucugugcgaccugcugaucaggugcaucaacugccagaagccccugugccccgaggagaagcagagacaccuggacaagaagcagagguuccacaauaccaggggccgcuggaccggccgcugcaugucuugcugcagguccagccggaccaggagagagacccagcuggccggagcacacggagauacacccacccugcacgaguacaugcuggaccugcagccugagaccaccgaccuguacugcgggaguggauacgaacagcugaacgacagcagcgaggaggaggacgagaucgacggccccgccggacaggcugagccugauagggcccacuacaacauugugacauuuugcugcaagugcgacagcacccugaggcugugcgugcagagcacccacguggauaucaggacccuggaggaucugcugaugggaacccugggcaucgugugccccaucugcucccagaagccugacuacaaggacgacgacgacaag

SEQ ID NO: 14 - RNA, 807 nt, Artificial sequence
  fusion protein in plasmid pVR-E6E7
augcaccagaagaggacagcaauguuccaggacccacaggagaggccaaggaagcugccacagcugugcacagagcugcagacaacaauccacgauauuauccuggagugcguguauugcaagcagcagcugcugaggagggagguguaugacuucgcuuucagagaccuguguaucguguaccgggacgggaacccuuacgcagugggcgacaagugccugaaguucuauagcaagaucagcgaguacaggcacuacuguuacagccuguauggaaccacccuggagcagcaguauaacaaaccucugugcgaccugcugaucaggugcaucaacugccagaagccccugugccccgaggagaagcagagacaccuggacaagaagcagagguuccacaauaccaggggccgcuggaccggccgcugcaugucuugcugcagguccagccggaccaggagagagacccagcuggccggagcacacggagauacacccacccugcacgaguacaugcuggaccugcagccugagaccaccgaccuguacugcgggaguggauacgaacagcugaacgacagcagcgaggaggaggacgagaucgacggccccgccggacaggcugagccugauagggcccacuacaacauugugacauuuugcugcaagugcgacagcacccugaggcugugcgugcagagcacccacguggauaucaggacccuggaggaucugcugaugggaacccugggcaucgugugccccaucugcucccagaagccugacuacaaggacgacgacgacaag

SEQ ID NO: 15 - protein, 402 aa, Artificial sequence
  fusion protein in plasmid pVR-CCL11-E6E7-T2
MDWTWILFLVAAATRVHSGPASVPTTCCFNLANRKIPLQRLESYRRITSGKCPQKAVIFKTKLAKDICADPKKKWVQDSMKYLDQKSPTPKPGGGGGSGGGGGHQKRTAMFQDPQERPRKLPQLCTELQTTIHDIILECVYCKQQLLRREVYDFAFRDLCIVYRDGNPYAVGDKCLKFYSKISEYRHYCYSLYGTTLEQQYNKPLCDLLIRCINCQKPLCPEEKQRHLDKKQRFHNTRGRWTGRCMSCCRSSRTRRETQLAGAHGDTPTLHEYMLDLQPETTDLYCGSGYEQLNDSSEEEDEIDGPAGQAEPDRAHYNIVTFCCKCDSTLRLCVQSTHVDIRTLEDLLMGTLGIVCPICSQKPPGSGYIPEAPRDGQAYVRKDGEWVLLSTFLGDYKDDDDK

SEQ ID NO: 16 - protein, 371 aa, Artificial sequence
  fusion protein in plasmid pVR-CCL11-E6E7
MDWTWILFLVAAATRVHSGPASVPTTCCFNLANRKIPLQRLESYRRITSGKCPQKAVIFKTKLAKDICADPKKKWVQDSMKYLDQKSPTPKPGGGGGSGGGGGHQKRTAMFQDPQERPRKLPQLCTELQTTIHDIILECVYCKQQLLRREVYDFAFRDLCIVYRDGNPYAVGDKCLKFYSKISEYRHYCYSLYGTTLEQQYNKPLCDLLIRCINCQKPLCPEEKQRHLDKKQRFHNTRGRWTGRCMSCCRSSRTRRETQLAGAHGDTPTLHEYMLDLQPETTDLYCGSGYEQLNDSSEEEDEIDGPAGQAEPDRAHYNIVTFCCKCDSTLRLCVQSTHVDIRTLEDLLMGTLGIVCPICSQKPDYKDDDDK

SEQ ID NO: 17 - protein, 269 aa, Artificial sequence
  fusion protein in plasmid pVR-E6E7
MHQKRTAMFQDPQERPRKLPQLCTELQTTIHDIILECVYCKQQLLRREVYDFAFRDLCIVYRDGNPYAVGDKCLKFYSKISEYRHYCYSLYGTTLEQQYNKPLCDLLIRCINCQKPLCPEEKQRHLDKKQRFHNTRGRWTGRCMSCCRSSRTRRETQLAGAHGDTPTLHEYMLDLQPETTDLYCGSGYEQLNDSSEEEDEIDGPAGQAEPDRAHYNIVTFCCKCDSTLRLCVQSTHVDIRTLEDLLMGTLGIVCPICSQKPDYKDDDDK